European Patent Application EP 4 186 529 A1, published May 31, 2023. Title: Improved Antibody-Payload Conjugates (APCs) prepared by site-specific conjugation utilizing genetic code expansion. Applicant: Veraxa Biotech GmbH. Application EP. The sequence listing filed with the application follows.

SEQUENCE LISTING (116 sequences)

SEQ ID NO: 1 - DNA, 1350 bp, synthetic construct
  misc_feature 1..1350: note = Trastuzumab Heavy Chain
  source 1..1350: mol_type = other DNA
gaagtgcagctggtcgagtccggtggtggcctggttcagcctggtggttccctgcgtctgtcctgcgctgcttccggtttcaacatcaaggacacctacatccactgggtccgccaggctcccggcaagggattggaatgggtggcccgtatctaccccaccaacggttacacccgttacgctgactccgtgaagggccgtttcaccatctccgctgacacctccaagaacaccgcttacctgcagatgaactccctgcgtgctgaggacaccgctgtgtactactgctcccgttggggtggcgacggtttctacgctatggactactggggccagggcaccctggtcaccgtgtcctctgcttccaccaagggcccctccgtgttccctctggctccatcctccaagtccacctccggtggaaccgctgctctgggttgcctggtcaaggactacttccccgagcccgtgaccgtgtcttggaactccggtgctctgacctccggcgtgcacaccttccctgctgtcctgcagtcctccggcctgtactccctgtcctccgtcgtgactgtgccctcatcctccctgggcacccagacctacatctgcaacgtgaaccacaagccctccaacaccaaggtggacaagaaggtcgagcccaagtcctgcgacaagacccacacttgccccccttgccctgctcctgaactgctcggtggcccctccgtgtttctgttccctcccaagcccaaggacaccctgatgatctcccgcactcccgaggtgacttgcgtcgtggtggatgtgtcccacgaggaccccgaggtgaagttcaactggtacgtggacggcgtcgaggtgcacaacgctaagaccaagccccgtgaggagcagtacaacagcacctaccgcgtcgtgtccgtgctcaccgtgctgcaccaggactggctgaacggcaaggagtacaagtgcaaagtgtccaacaaggccctgcccgctcccatcgagaagaccatctccaaggctaagggccaacctcgtgagccccaggtgtacactctgcctcccagccgcgaggagatgaccaagaaccaggtctccctcacctgcctggtgaaaggcttctacccctccgacatcgccgtggaatgggagagcaacggccagcccgagaacaactacaagaccacccctcccgtgctggactccgacggttccttcttcctgtacagcaagctgaccgtggacaagtcccgttggcagcagggcaacgtgttctcctgctccgtgatgcacgaggccctgcacaatcactacactcagaagtccctgtccctgtcccccggcaag

SEQ ID NO: 2 - protein, 450 aa, synthetic construct
  REGION 1..450: note = Synthetic Construct
EVQLVESGGGLVQPGGSLRLSCAASGFNIKDTYIHWVRQAPGKGLEWVARIYPTNGYTRYADSVKGRFTISADTSKNTAYLQMNSLRAEDTAVYYCSRWGGDGFYAMDYWGQGTLVTVSSASTKGPSVFPLAPSSKSTSGGTAALGCLVKDYFPEPVTVSWNSGALTSGVHTFPAVLQSSGLYSLSSVVTVPSSSLGTQTYICNVNHKPSNTKVDKKVEPKSCDKTHTCPPCPAPELLGGPSVFLFPPKPKDTLMISRTPEVTCVVVDVSHEDPEVKFNWYVDGVEVHNAKTKPREEQYNSTYRVVSVLTVLHQDWLNGKEYKCKVSNKALPAPIEKTISKAKGQPREPQVYTLPPSREEMTKNQVSLTCLVKGFYPSDIAVEWESNGQPENNYKTTPPVLDSDGSFFLYSKLTVDKSRWQQGNVFSCSVMHEALHNHYTQKSLSLSPGK

SEQ ID NO: 3 - DNA, 642 bp, synthetic construct
  misc_feature 1..642: note = Trastuzumab light chain
  source 1..642: mol_type = other DNA
gacatccagatgacccagtccccctcctccctgtccgcttccgtgggagatcgtgtgaccatcacttgccgtgcttcccaggacgtgaacaccgctgtggcttggtaccagcagaagcccggcaaggctcccaagctgctgatctactccgctagcttcctgtactccggtgtcccctcccgtttctccggttcccgttccggtactgacttcaccctgaccatctccagcctgcagcccgaggacttcgctacctactactgccagcagcactacaccaccccccccaccttcggccagggtactaaggtcgagatcaagcgtaccgtggctgctccctccgtgttcatcttcccaccctccgacgagcagctgaagtccggcactgcttccgtcgtgtgcctgctgaacaacttctacccccgcgaggctaaggtgcagtggaaggtggacaacgctctgcagtccggcaactcccaagagtccgtgaccgagcaggactccaaggactctacctactctctgtcctctaccctgaccctgtccaaggctgactacgagaagcacaaggtgtacgcttgcgaagtgacccaccagggcctgtcctccccagtgaccaagtccttcaaccgtggcgagtgc

SEQ ID NO: 4 - protein, 214 aa, synthetic construct
  REGION 1..214: note = Synthetic Construct
DIQMTQSPSSLSASVGDRVTITCRASQDVNTAVAWYQQKPGKAPKLLIYSASFLYSGVPSRFSGSRSGTDFTLTISSLQPEDFATYYCQQHYTTPPTFGQGTKVEIKRTVAAPSVFIFPPSDEQLKSGTASVVCLLNNFYPREAKVQWKVDNALQSGNSQESVTEQDSKDSTYSLSSTLTLSKADYEKHKVYACEVTHQGLSSPVTKSFNRGEC

SEQ ID NO: 5 - DNA, 1344 bp, synthetic construct
  misc_feature 1..1344: note = Pertuzumab Heavy chain
  source 1..1344: mol_type = other DNA
gaggtgcagctggtggagagcggaggcggcttggtacagcctggcgggagtctgagactgagctgcgccgcaagcggcttcaccttcaccgactacaccatggactgggtgagacaagcccccggcaagggcctggagtgggtggccgacgtgaaccccaacagcggcggcagcatctacaatcagagattcaagggcagattcaccctgagcgtggacagaagcaagaacaccctgtacctgcagatgaacagcctgagagccgaggacaccgccgtgtactactgcgctagaaacctgggccctagcttctacttcgactactggggccaaggcaccctggtaaccgttagcagcgcaagcacaaaaggtcctagcgtgttccctttagccccctctagcaagagcacaagcggcggtacagcggccctgggctgcctagtgaaggattattttccggaacccgtgaccgtcagttggaattccggcgcactgacaagcggcgttcacaccttccccgccgtgctgcagagcagcggcctgtacagcctgagcagcgtggtgaccgtgcctagcagcagcctgggcacacagacctacatctgcaacgtgaaccacaagcctagcaacaccaaggtggacaagaaggtggagccgaagagctgtgacaagacccacacctgccccccctgccccgcccccgaactgctgggcggaccctccgtgttcctttttccccccaagcccaaggacaccctgatgatcagcagaacccccgaggtgacctgcgtggtggtggacgtgagccacgaggaccccgaggtgaagttcaactggtacgtggacggcgtggaggtgcacaacgccaagaccaagcctagagaggagcagtacaacagcacctacagagtggtgagcgtgctgaccgtgctgcaccaagactggctgaacggcaaggagtacaagtgcaaggtgagcaacaaggccctgcccgcccccatcgagaagaccatcagcaaggccaaggggcagcctagagagccccaagtgtacaccctgccccctagcagagaggagatgaccaagaaccaagtgagcctgacctgcctggtgaaggggttttaccctagcgacatcgccgtggagtgggagagcaacgggcagcccgagaacaactacaagaccaccccccccgtgctggacagcgacggcagcttcttcctgtacagcaagctgaccgtggacaagagcagatggcagcaaggcaacgtgttcagctgcagcgtgatgcacgaggccctgcacaaccactacacacagaagagcctgagcctgagccccggc

SEQ ID NO: 6 - protein, 448 aa, synthetic construct
  REGION 1..448: note = Synthetic Construct
EVQLVESGGGLVQPGGSLRLSCAASGFTFTDYTMDWVRQAPGKGLEWVADVNPNSGGSIYNQRFKGRFTLSVDRSKNTLYLQMNSLRAEDTAVYYCARNLGPSFYFDYWGQGTLVTVSSASTKGPSVFPLAPSSKSTSGGTAALGCLVKDYFPEPVTVSWNSGALTSGVHTFPAVLQSSGLYSLSSVVTVPSSSLGTQTYICNVNHKPSNTKVDKKVEPKSCDKTHTCPPCPAPELLGGPSVFLFPPKPKDTLMISRTPEVTCVVVDVSHEDPEVKFNWYVDGVEVHNAKTKPREEQYNSTYRVVSVLTVLHQDWLNGKEYKCKVSNKALPAPIEKTISKAKGQPREPQVYTLPPSREEMTKNQVSLTCLVKGFYPSDIAVEWESNGQPENNYKTTPPVLDSDGSFFLYSKLTVDKSRWQQGNVFSCSVMHEALHNHYTQKSLSLSPG

SEQ ID NO: 7 - DNA, 642 bp, synthetic construct
  misc_feature 1..642: note = PertuzumabLight chain
  source 1..642: mol_type = other DNA
gacattcagatgacacagagccctagcagcctgagcgcaagcgtgggcgacagagtgaccatcacctgcaaggcaagccaagacgtgagcatcggcgtggcctggtatcagcagaagcccggcaaggcccccaagctgctgatctacagcgcaagctacagatacaccggcgtgcctagcagattcagcggcagcggcagcggcaccgacttcaccctgaccatcagcagcctgcagcccgaggacttcgccacctactactgtcagcagtactacatctacccctacaccttcggccaaggcaccaaggtggagatcaagagaaccgtggccgcccctagcgtgttcatcttcccccctagcgacgagcagctgaagagcggcaccgcaagcgtggtgtgcctgctgaacaacttctaccctagagaggccaaggtgcagtggaaggtggacaacgccctgcagagcggcaacagccaagagagcgtgaccgagcaagacagcaaggacagcacctacagcctgagcagcaccctgaccctgagcaaggccgactacgagaagcacaaggtgtacgcctgcgaggtgacccaccaaggcctgagcagccccgtgaccaagagcttcaacagaggcgagtgc

SEQ ID NO: 8 - protein, 214 aa, synthetic construct
  REGION 1..214: note = Synthetic Construct
DIQMTQSPSSLSASVGDRVTITCKASQDVSIGVAWYQQKPGKAPKLLIYSASYRYTGVPSRFSGSGSGTDFTLTISSLQPEDFATYYCQQYYIYPYTFGQGTKVEIKRTVAAPSVFIFPPSDEQLKSGTASVVCLLNNFYPREAKVQWKVDNALQSGNSQESVTEQDSKDSTYSLSSTLTLSKADYEKHKVYACEVTHQGLSSPVTKSFNRGEC

SEQ ID NO: 9 - protein, 10 aa, synthetic construct
  REGION 1..10: note = Trastuzumab CDR-H1
GFNIKDTYIH

SEQ ID NO: 10 - protein, 8 aa, synthetic construct
  REGION 1..8: note = Pertuzumab CDR-H1
GFTFTDYT

SEQ ID NO: 11 - protein, 11 aa, synthetic construct
  REGION 1..11: note = Trastuzumab CDR-H2
ARIYPTNGYTR

SEQ ID NO: 12 - protein, 8 aa, synthetic construct
  REGION 1..8: note = Pertuzumab CDR-H2
VNPNSGGS

SEQ ID NO: 13 - protein, 13 aa, synthetic construct
  REGION 1..13: note = Trastuzumab CDR-H3
SRWGGDGFYAMDY

SEQ ID NO: 14 - protein, 11 aa, synthetic construct
  REGION 1..11: note = Pertuzumab CDR-H3
RNLGPSFYFDY

SEQ ID NO: 15 - protein, 6 aa, synthetic construct
  REGION 1..6: note = Trastuzumab CDR-L1
QDVNTA

SEQ ID NO: 16 - protein, 5 aa, synthetic construct
  REGION 1..5: note = Pertuzumab CDR-L1
DVSIG

SEQ ID NO: 17-18 - skipped (2 entries)

SEQ ID NO: 19 - protein, 8 aa, synthetic construct
  REGION 1..8: note = Trastuzumab CDR-L3
QQHYTTPP

SEQ ID NO: 20 - protein, 8 aa, synthetic construct
  REGION 1..8: note = Pertuzumab CDR-L3
QQYYIYPY

SEQ ID NO: 21 - DNA, 4412 bp, synthetic construct
  misc_feature 1..4412: note = Plasmid
  source 1..4412: mol_type = other DNA
ttctctgtcacagaatgaaaatttttctgtcatctcttcgttattaatgtttgtaattgactgaatatcaacgcttatttgcagcctgaatggcgaatgggacgcgccctgtagcggcgcattaagcgcggcgggtgtggtggttacgcgcagcgtgaccgctacacttgccagcgccctagcgcccgctcctttcgctttcttcccttcctttctcgccacgttcgccgcaaactattaactggcgaactacttactctagcttcccggcaacaattaatagactggatggaggcggataaagttgcaggaccacttctgcgctcggcccttccggctggctggtttattgctgataaatctggagccggtgagcgtgggtctcgcggtatcattgcagcactggggccagatggtaagccctcccgtatcgtagttatctacacgacggggagtcaggcaactatggatgaacgaaatagacagatcgctgagataggtgcctcactgattaagcattggtaactgtcagaccaagtttactcatatatactttagattgatttaaaacttcatttttaatttaaaaggatctaggtgaagatcctttttgataatctcatgaccaaaatcccttaacgtgagttttcgttccactgagcgtcagaccccgtagaaaagatcaaaggatcttcttgagatcctttttttctgcgcgtaatctgctgcttgcaaacaaaaaaaccaccgctaccagcggtggtttgtttgccggatcaagagctaccaactctttttccgaaggtaactggcttcagcagagcgcagataccaaatactgttcttctagtgtagccgtagttaggccaccacttcaagaactctgtagcaccgcctacatacctcgctctgctaatcctgttaccagtggctgctgccagtggcgataagtcgtgtcttaccgggttggactcaagacgatagttaccggataaggcgcagcggtcgggctgaacggggggttcgtgcacacagcccagcttggagcgaacgacctacaccgaactgagatacctacagcgtgagctatgagaaagcgccacgcttcccgaagggagaaaggcggacaggtatccggtaagcggcagggtcggaacaggagagcgcacgagggagcttccagggggaaacgcctggtatctttatagtcctgtcgggtttcgccacctctgacttgagcgtcgatttttgtgatgctcgtcaggggggcggagcctatggaaaaacgccagcaacgcggcctttttacggttcctggccttttgctggccttttgctcacatgttctttcctgcgttatcccctgattctgtggataaccgtattaccgcctttgagtgagctgataccgctcgccgcagccgaacgaccgagcgcagcgagtcagtgagcgaggaagcggaagagcgcctgatgcggtattttctccttacgcatctgtgcggtatttcacaccgcatagaccagccgcgtaacctggcaaaatcggttacggttgagtaataaatggatgccctgcgtaagcgggtgtgggcggacaataaagtcttaaactgaacaaaatagatctaaactatgacaataaagtcttaaactagacagaatagttgtaaactgaaatcagtccagttatgctgtgaaaaagcatactggacttttgttatggctaaagcaaactcttcattttctgaagtgcaaattgcccgtcgtattaaagaggggcgtggccaagggcatggtaaagactatattcgcggcgttgtgacaatttaccgaacaactccgcggccgggaagccgatctcggcttgaacgaattgttaggtggcggtacttgggtcgatatcaaagtgcatcacttcttcccgtatgcccaactttgtatagagagccactgcgggatcgtcaccgtaatctgcttgcacgtagatcacataagcaccaagcgcgttggcctcatgcttgaggagattgatgagcgcggtggcaatgccctgcctccggtgctcgccggagactgcgagatcatagatatagatctcactacgcggctgctcaaacttgggcagaacgtaagccgcgagagcgccaacaaccgcttcttggtcgaaggcagcaagcgcgatgaatgtcttactacggagcaagttcccgaggtaatcggagtccggctgatgttgggagtaggtggctacgtctccgaactcacgaccgaaaagatcaagagcagcccgcatggatttgacttggtcagggccgagcctacatgtgcgaatgatgcccatacttgagccacctaactttgttttagggcgactgccctgctgcgtaacatcgttgctgctgcgtaacatcgttgctgctccataacatcaaacatcgacccacggcgtaacgcgcttgctgcttggatgcccgaggcatagactgtacaaaaaaacagtcataacaagccatgaaaaccgccactgcgccgttaccaccgctgcgttcggtcaaggttctggaccagttgcgtgagcgcatacgctacttgcattacagtttacgaaccgaacaggcttatgtcaactgggttcgtgccttcatccgtttccacggtgtgcgtcacccggcaaccttgggcagcagcgaagtcgaggcatttctgtcctggctggcgaacgagcgcaaggtttcggtctccacgcatcgtcaggcattggcggccttgctgttcttctacggcaaggtgctgtgcacggatctgcccttgcttcaggagatcggtagacctcggccgtcgcggcgcttgccggtggtgctgaccccggatgaagtggttcgcatcctcggttttctggaaggcgagcatcgtttgttcgcccaggactctagctatagttctagtggttggctacagctttgtttgtactatcaacaggttgaactgctgatcaacagatcctctacgcggccgcggtaccataacttcgtatagcatacattatacgaagttatctggtttaaacgtacccgtagtggctatggcagggcttgccgccccgacgttggctgcgagccctgggccttcacccgaacttgggggttggggtggggaaaaggaagaaacgcgggcgtattggtcccaatggggtctcggtggggtatcgacagagtgccagccctgggaccgaaccccgcgtttatgaacaaacgacccaacacccgtgcgttttattctgtctttttattgccgtcatagcgcgggttccttccggtattgtctccttccgtgtttcagttagcctcccccatctcccggtaccgcatgctatgcatcagctgctagcaccatggctcgagatcccgggtgatcaagtcttcgtcgagtgattgtaaataaaatgtaatttacagtatagtattttaattaatatacaaatgatttgataataattcttatttaactataatatattgtgttgggttgaattaaaggtccgtacgacctactccggaatattaatagatcatggagataattaaaatgataaccatctcgcaaataaataagtattttactgttttcgtaacagttttgtaataaaaaaacctataaatattccggattattcataccgtcccaccatcgggcgcggatcccggtccgaagcgcgcggaattcaaaggcctacgtcgacgagctcactagtcgcggccgctttcgaatctagagcctgcagtctcgacaagcttgtcgagaagtactagaggatcataatcagccataccacatttgtagaggttttacttgctttaaaaaacctcccacacctccccctgaacctgaaacataaaatgaatgcaattgttgttgttaacttgtttattgcagcttataatggttacaaataaagcaatagcatcacaaatttcacaaataaagcatttttttcactgcattctagttgtggtttgtccaaactcatcaatgtatcttatcatgtctggatctgatcactgcttgagcctagaagatccggctgctaacaaagcccgaaaggaagctgagttggctgctgccaccgctgagcaataactatcataacccctaggagatccgaaccagataagtgaaatctagttccaaactattttgtcatttttaattttcgtattagcttacgacgctacacccagttcccatctattttgtcactcttccctaaataatccttaaaaactccatttccacccctcccagttcccaactattttgtccgcccacagcggggcatttttcttcctgttatgtttttaatcaaacatcctgccaactccatgtgacaaaccgtcatcttcggctacttt

SEQ ID NO: 22 - DNA, 6401 bp, synthetic construct
  misc_feature 1..6401: note = Plasmid
  source 1..6401: mol_type = other DNA
tattaatattccggagtaggtcgcggacctttaattcaacccaacacaatatattatagttaaataagaattattatcaaatcatttgtatattaattaaaatactatactgtaaattacattttatttacaatcactcgacgaagacttgatcacccgggatggaagtgcagctggtcgagtccggtggtggcctggttcagcctggtggttccctgcgtctgtcctgcgctgcttccggtttcaacatcaaggacacctacatccactgggtccgccaggctcccggcaagggattggaatgggtggcccgtatctaccccaccaacggttacacccgttacgctgactccgtgaagggccgtttcaccatctccgctgacacctccaagaacaccgcttacctgcagatgaactccctgcgtgctgaggacaccgctgtgtactactgctcccgttggggtggcgacggtttctacgctatggactactggggccagggcaccctggtcaccgtgtcctctgcttccaccaagggcccctccgtgttccctctggctccatcctccaagtccacctccggtggaaccgctgctctgggttgcctggtcaaggactacttccccgagcccgtgaccgtgtcttggaactccggtgctctgacctccggcgtgcacaccttccctgctgtcctgcagtcctccggcctgtactccctgtcctccgtcgtgactgtgccctcatcctccctgggcacccagacctacatctgcaacgtgaaccacaagccctccaacaccaaggtggacaagaaggtcgagcccaagtcctgcgacaagacccacacttgccccccttgccctgctcctgaactgctcggtggcccctccgtgtttctgttccctcccaagcccaaggacaccctgatgatctcccgcactcccgaggtgacttgcgtcgtggtggatgtgtcccacgaggaccccgaggtgaagttcaactggtacgtggacggcgtcgaggtgcacaacgctaagaccaagccccgtgaggagcagtacaacagcacctaccgcgtcgtgtccgtgctcaccgtgctgcaccaggactggctgaacggcaaggagtacaagtgcaaagtgtccaacaaggccctgcccgctcccatcgagaagaccatctccaaggctaagggccaacctcgtgagccccaggtgtacactctgcctcccagccgcgaggagatgaccaagaaccaggtctccctcacctgcctggtgaaaggcttctacccctccgacatcgccgtggaatgggagagcaacggccagcccgagaacaactacaagaccacccctcccgtgctggactccgacggttccttcttcctgtacagcaagctgaccgtggacaagtcccgttggcagcagggcaacgtgttctcctgctccgtgatgcacgaggccctgcacaatcactacactcagaagtccctgtccctgtcccccggcaagcatcaccatcaccaccactaagctagcagctgatgcatagcatgcggtaccgggagatgggggaggctaactgaaacacggaaggagacaataccggaaggaacccgcgctatgacggcaataaaaagacagaataaaacgcacgggtgttgggtcgtttgttcataaacgcggggttcggtcccagggctggcactctgtcgataccccaccgagaccccattgggaccaatacgcccgcgtttcttccttttccccaccccaacccccaagttcgggtgaaggcccagggctcgcagccaacgtcggggcggcaagccctgccatagccactacgggtacgtttaaaccagataacttcgtataatgtatgctatacgaagttatggtaccgcggccgcgtagaggatctgttgatcagcagttcaacctgttgatagtacaaacaaagctgtagccaaccactagaactatagctagagtcctgggcgaacaaacgatgctcgccttccagaaaaccgaggatgcgaaccacttcatccggggtcagcaccaccggcaagcgccgcgacggccgaggtctaccgatctcctgaagcaagggcagatccgtgcacagcaccttgccgtagaagaacagcaaggccgccaatgcctgacgatgcgtggagaccgaaaccttgcgctcgttcgccagccaggacagaaatgcctcgacttcgctgctgcccaaggttgccgggtgacgcacaccgtggaaacggatgaaggcacaaacccagttgacataagcctgttcggttcgtaaactgtaatgcaagtagcgtatgcgctcacgcaactggtccagaaccttgaccgaacgcagcggtggtaacggcgcagtggcggttttcatggcttgttatgactgtttttttgtacagtctatgcctcgggcatccaagcagcaagcgcgttacgccgtgggtcgatgtttgatgttatggagcagcaacgatgttacgcagcagcaacgatgttacgcagcagggcagtcgccctaaaacaaagttaggtggctcaagtatgggcatcattcgcacatgtaggctcggccctgaccaagtcaaatccatgcgggctgctcttgatcttttcggtcgtgagttcggagacgtagccacctactcccaacatcagccggactccgattacctcgggaacttgctccgtagtaagacattcatcgcgcttgctgccttcgaccaagaagcggttgttggcgctctcgcggcttacgttctgcccaagtttgagcagccgcgtagtgagatctatatctatgatctcgcagtctccggcgagcaccggaggcagggcattgccaccgcgctcatcaatctcctcaagcatgaggccaacgcgcttggtgcttatgtgatctacgtgcaagcagattacggtgacgatcccgcagtggctctctatacaaagttgggcatacgggaagaagtgatgcactttgatatcgacccaagtaccgccacctaacaattcgttcaagccgagatcggcttcccggccgcggagttgttcggtaaattgtcacaacgccgcgaatatagtctttaccatgcccttggccacgcccctctttaatacgacgggcaatttgcacttcagaaaatgaagagtttgctttagccataacaaaagtccagtatgctttttcacagcataactggactgatttcagtttacaactattctgtctagtttaagactttattgtcatagtttagatctattttgttcagtttaagactttattgtccgcccacacccgcttacgcagggcatccatttattactcaaccgtaaccgattttgccaggttacgcggctggtctatgcggtgtgaaataccgcacagatgcgtaaggagaaaataccgcatcaggcgctcttccgcttcctcgctcactgactcgctgcgctcggtcgttcggctgcggcgagcggtatcagctcactcaaaggcggtaatacggttatccacagaatcaggggataacgcaggaaagaacatgtgagcaaaaggccagcaaaaggccaggaaccgtaaaaaggccgcgttgctggcgtttttccataggctccgcccccctgacgagcatcacaaaaatcgacgctcaagtcagaggtggcgaaacccgacaggactataaagataccaggcgtttccccctggaagctccctcgtgcgctctcctgttccgaccctgccgcttaccggatacctgtccgcctttctcccttcgggaagcgtggcgctttctcatagctcacgctgtaggtatctcagttcggtgtaggtcgttcgctccaagctgggctgtgtgcacgaaccccccgttcagcccgaccgctgcgccttatccggtaactatcgtcttgagtccaacccggtaagacacgacttatcgccactggcagcagccactggtaacaggattagcagagcgaggtatgtaggcggtgctacagagttcttgaagtggtggcctaactacggctacactagaagaacagtatttggtatctgcgctctgctgaagccagttaccttcggaaaaagagttggtagctcttgatccggcaaacaaaccaccgctggtagcggtggtttttttgtttgcaagcagcagattacgcgcagaaaaaaaggatctcaagaagatcctttgatcttttctacggggtctgacgctcagtggaacgaaaactcacgttaagggattttggtcatgagattatcaaaaaggatcttcacctagatccttttaaattaaaaatgaagttttaaatcaatctaaagtatatatgagtaaacttggtctgacagttaccaatgcttaatcagtgaggcacctatctcagcgatctgtctatttcgttcatccatagttgcctgactccccgtcgtgtagataactacgatacgggagggcttaccatctggccccagtgctgcaatgataccgcgagacccacgctcaccggctccagatttatcagcaataaaccagccagccggaagggccgagcgcagaagtggtcctgcaactttatccgcctccatccagtctattaattgttgccgggaagctagagtaagtagttcgccagttaatagtttgcggcgaacgtggcgagaaaggaagggaagaaagcgaaaggagcgggcgctagggcgctggcaagtgtagcggtcacgctgcgcgtaaccaccacacccgccgcgcttaatgcgccgctacagggcgcgtcccattcgccattcaggctgcaaataagcgttgatattcagtcaattacaaacattaataacgaagagatgacagaaaaattttcattctgtgacagagaaaaagtagccgaagatgacggtttgtcacatggagttggcaggatgtttgattaaaaacataacaggaagaaaaatgccccgctgtgggcggacaaaatagttgggaactgggaggggtggaaatggagtttttaaggattatttagggaagagtgacaaaatagatgggaactgggtgtagcgtcgtaagctaatacgaaaattaaaaatgacaaaatagtttggaactagatttcacttatctggttcggatctcctaggggttatgatagttattgctcagcggtggcagcagccaactcagcttcctttcgggctttgttagcagccggatcttctaggctcaagcagtgatcagatccagacatgataagatacattgatgagtttggacaaaccacaactagaatgcagtgaaaaaaatgctttatttgtgaaatttgtgatgctattgctttatttgtaaccattataagctgcaataaacaagttaacaacaacaattgcattcattttatgtttcaggttcagggggaggtgtgggaggttttttaaagcaagtaaaacctctacaaatgtggtatggctgattatgatcctctagtacttctcgacaagcttgtcgagactgcaggctctagattcgaaagcggccgcgactagtgagctcgtcgacgtaggcctttgaattcttagcactcgccacggttgaaggacttggtcactggggaggacaggccctggtgggtcacttcgcaagcgtacaccttgtgcttctcgtagtcagccttggacagggtcagggtagaggacagagagtaggtagagtccttggagtcctgctcggtcacggactcttgggagttgccggactgcagagcgttgtccaccttccactgcaccttagcctcgcgggggtagaagttgttcagcaggcacacgacggaagcagtgccggacttcagctgctcgtcggagggtgggaagatgaacacggagggagcagccacggtacgcttgatctcgaccttagtaccctggccgaaggtggggggggtggtgtagtgctgctggcagtagtaggtagcgaagtcctcgggctgcaggctggagatggtcagggtgaagtcagtaccggaacgggaaccggagaaacgggaggggacaccggagtacaggaagctagcggagtagatcagcagcttgggagccttgccgggcttctgctggtaccaagccacagcggtgttcacgtcctgggaagcacggcaagtgatggtcacacgatctcccacggaagcggacagggaggagggggactgggtcatctggatgtccatggatccgcgcccgatggtgggacggtatgaataatccggaatatttataggtttttttattacaaaactgttacgaaaacagtaaaatacttatttatttgcgagatggttatcattttaattatctccatgatc

SEQ ID NO: 23 - DNA, 31 bp, synthetic construct
  misc_feature 1..31: note = PCR primer
  source 1..31: mol_type = other DNA
caggcttagggcaagggattggaatgggtgg

SEQ ID NO: 24 - DNA, 25 bp, synthetic construct
  misc_feature 1..25: note = PCR primer
  source 1..25: mol_type = other DNA
cttgccctaagcctggcggacccag

SEQ ID NO: 25 - DNA, 30 bp, synthetic construct
  misc_feature 1..30: note = PCR primer
  source 1..30: mol_type = other DNA
gctccctagaagggattggaatgggtggcc

SEQ ID NO: 26 - DNA, 24 bp, synthetic construct
  misc_feature 1..24: note = PCR primer
  source 1..24: mol_type = other DNA
tcccttctagggagcctggcggac

SEQ ID NO: 27 - DNA, 30 bp, synthetic construct
  misc_feature 1..30: note = PCR primer
  source 1..30: mol_type = other DNA
cctccctagcccaaggacaccctgatgatc

SEQ ID NO: 28 - DNA, 30 bp, synthetic construct
  misc_feature 1..30: note = PCR primer
  source 1..30: mol_type = other DNA
tgggctagggagggaacagaaacacggagg

SEQ ID NO: 29 - DNA, 29 bp, synthetic construct
  misc_feature 1..29: note = PCR primer
  source 1..29: mol_type = other DNA
aagccctaggacaccctgatgatctcccg

SEQ ID NO: 30 - DNA, 29 bp, synthetic construct
  misc_feature 1..29: note = PCR primer
  source 1..29: mol_type = other DNA
tgtcctagggcttgggagggaacagaaac

SEQ ID NO: 31 - DNA, 38 bp, synthetic construct
  misc_feature 1..38: note = PCR primer
  source 1..38: mol_type = other DNA
aacggctaggagtacaagtgcaaagtgtccaacaaggc

SEQ ID NO: 32 - DNA, 28 bp, synthetic construct
  misc_feature 1..28: note = PCR primer
  source 1..28: mol_type = other DNA
gtactcctagccgttcagccagtcctgg

SEQ ID NO: 33 - DNA, 27 bp, synthetic construct
  misc_feature 1..27: note = PCR primer
  source 1..27: mol_type = other DNA
aaggcttagggccaacctcgtgagccc

SEQ ID NO: 34 - DNA, 34 bp, synthetic construct
  misc_feature 1..34: note = PCR primer
  source 1..34: mol_type = other DNA
ttggccctaagccttggagatggtcttctcgatg

SEQ ID NO: 35 - DNA, 30 bp, synthetic construct
  misc_feature 1..30: note = PCR primer
  source 1..30: mol_type = other DNA
aagccctagaaggctcccaagctgctgatc

SEQ ID NO: 36 - DNA, 30 bp, synthetic construct
  misc_feature 1..30: note = PCR primer
  source 1..30: mol_type = other DNA
agccttctagggcttctgctggtaccaagc

SEQ ID NO: 37 - DNA, 30 bp, synthetic construct
  misc_feature 1..30: note = PCR primer
  source 1..30: mol_type = other DNA
tactcctagagcttcctgtactccggtgtc

SEQ ID NO: 38 - DNA, 33 bp, synthetic construct
  misc_feature 1..33: note = PCR primer
  source 1..33: mol_type = other DNA
gaagctctaggagtagatcagcagcttgggagc

SEQ ID NO: 39 - DNA, 26 bp, synthetic construct
  misc_feature 1..26: note = PCR primer
  source 1..26: mol_type = other DNA
accacctagcccaccttcggccaggg

SEQ ID NO: 40 - DNA, 29 bp, synthetic construct
  misc_feature 1..29: note = PCR primer
  source 1..29: mol_type = other DNA
ggtgggctaggtggtgtagtgctgctggc

SEQ ID NO: 41 - DNA, 31 bp, synthetic construct
  misc_feature 1..31: note = PCR primer
  source 1..31: mol_type = other DNA
accgtgtaggctccctccgtgttcatcttcc

SEQ ID NO: 42 - DNA, 35 bp, synthetic construct
  misc_feature 1..35: note = PCR primer
  source 1..35: mol_type = other DNA
gggagcctacacggtacgcttgatctcgaccttag

SEQ ID NO: 43 - DNA, 36 bp, synthetic construct
  misc_feature 1..36: note = PCR primer
  source 1..36: mol_type = other DNA
gactcctaggactctacctactctctgtcctctacc

SEQ ID NO: 44 - DNA, 26 bp, synthetic construct
  misc_feature 1..26: note = PCR primer
  source 1..26: mol_type = other DNA
agtcctaggagtcctgctcggtcacg

SEQ ID NO: 45 - DNA, 1410 bp, synthetic construct
  misc_feature 1..1410: note = Secretion signal-modified Trastuzumab HC
  source 1..1410: mol_type = other DNA
atgaagtgggtaacctttatttcccttctttttctctttagctcggcttattccgaagtgcagctggtcgagtccggtggtggcctggttcagcctggtggttccctgcgtctgtcctgcgctgcttccggtttcaacatcaaggacacctacatccactgggtccgccaggctcccggcaagggattggaatgggtggcccgtatctaccccaccaacggttacacccgttacgctgactccgtgaagggccgtttcaccatctccgctgacacctccaagaacaccgcttacctgcagatgaactccctgcgtgctgaggacaccgctgtgtactactgctcccgttggggtggcgacggtttctacgctatggactactggggccagggcaccctggtcaccgtgtcctctgcttccaccaagggcccctccgtgttccctctggctccatcctccaagtccacctccggtggaaccgctgctctgggttgcctggtcaaggactacttccccgagcccgtgaccgtgtcttggaactccggtgctctgacctccggcgtgcacaccttccctgctgtcctgcagtcctccggcctgtactccctgtcctccgtcgtgactgtgccctcatcctccctgggcacccagacctacatctgcaacgtgaaccacaagccctccaacaccaaggtggacaagaaggtcgagcccaagtcctgcgacaagacccacacttgccccccttgccctgctcctgaactgctcggtggcccctccgtgtttctgttccctcccaagcccaaggacaccctgatgatctcccgcactcccgaggtgacttgcgtcgtggtggatgtgtcccacgaggaccccgaggtgaagttcaactggtacgtggacggcgtcgaggtgcacaacgctaagaccaagccccgtgaggagcagtacaacagcacctaccgcgtcgtgtccgtgctcaccgtgctgcaccaggactggctgaacggcaaggagtacaagtgcaaagtgtccaacaaggccctgcccgctcccatcgagaagaccatctccaaggctaagggccaacctcgtgagccccaggtgtacactctgcctcccagccgcgaggagatgaccaagaaccaggtctccctcacctgcctggtgaaaggcttctacccctccgacatcgccgtggaatgggagagcaacggccagcccgagaacaactacaagaccacccctcccgtgctggactccgacggttccttcttcctgtacagcaagctgaccgtggacaagtcccgttggcagcagggcaacgtgttctcctgctccgtgatgcacgaggccctgcacaatcactacactcagaagtccctgtccctgtcccccggcaagctaagc

SEQ ID NO: 46 - protein, 470 aa, synthetic construct
  REGION 1..470: note = Synthetic Construct
MKWVTFISLLFLFSSAYSEVQLVESGGGLVQPGGSLRLSCAASGFNIKDTYIHWVRQAPGKGLEWVARIYPTNGYTRYADSVKGRFTISADTSKNTAYLQMNSLRAEDTAVYYCSRWGGDGFYAMDYWGQGTLVTVSSASTKGPSVFPLAPSSKSTSGGTAALGCLVKDYFPEPVTVSWNSGALTSGVHTFPAVLQSSGLYSLSSVVTVPSSSLGTQTYICNVNHKPSNTKVDKKVEPKSCDKTHTCPPCPAPELLGGPSVFLFPPKPKDTLMISRTPEVTCVVVDVSHEDPEVKFNWYVDGVEVHNAKTKPREEQYNSTYRVVSVLTVLHQDWLNGKEYKCKVSNKALPAPIEKTISKAKGQPREPQVYTLPPSREEMTKNQVSLTCLVKGFYPSDIAVEWESNGQPENNYKTTPPVLDSDGSFFLYSKLTVDKSRWQQGNVFSCSVMHEALHNHYTQKSLSLSPGKLS

SEQ ID NO: 47 - DNA, 696 bp, synthetic construct
  misc_feature 1..696: note = Secretion signal-modified Trastuzumab LC
  source 1..696: mol_type = other DNA
atgaagtgggtaacctttatttcccttctttttctctttagctcggcttattccgacatccagatgacccagtccccctcctccctgtccgcttccgtgggagatcgtgtgaccatcacttgccgtgcttcccaggacgtgaacaccgctgtggcttggtaccagcagaagcccggcaaggctcccaagctgctgatctactccgctagcttcctgtactccggtgtcccctcccgtttctccggttcccgttccggtactgacttcaccctgaccatctccagcctgcagcccgaggacttcgctacctactactgccagcagcactacaccaccccccccaccttcggccagggtactaaggtcgagatcaagcgtaccgtggctgctccctccgtgttcatcttcccaccctccgacgagcagctgaagtccggcactgcttccgtcgtgtgcctgctgaacaacttctacccccgcgaggctaaggtgcagtggaaggtggacaacgctctgcagtccggcaactcccaagagtccgtgaccgagcaggactccaaggactctacctactctctgtcctctaccctgaccctgtccaaggctgactacgagaagcacaaggtgtacgcttgcgaagtgacccaccagggcctgtcctccccagtgaccaagtccttcaaccgtggcgagtgc

SEQ ID NO: 48 - protein, 232 aa, synthetic construct
  REGION 1..232: note = Synthetic Construct
MKWVTFISLLFLFSSAYSDIQMTQSPSSLSASVGDRVTITCRASQDVNTAVAWYQQKPGKAPKLLIYSASFLYSGVPSRFSGSRSGTDFTLTISSLQPEDFATYYCQQHYTTPPTFGQGTKVEIKRTVAAPSVFIFPPSDEQLKSGTASVVCLLNNFYPREAKVQWKVDNALQSGNSQESVTEQDSKDSTYSLSSTLTLSKADYEKHKVYACEVTHQGLSSPVTKSFNRGEC

SEQ ID NO: 49 - DNA, 7386 bp, synthetic construct
  misc_feature 1..7386: note = Plasmid
  source 1..7386: mol_type = other DNA
gacgtcaggtggcacttttcggggaaatgtgcgcggaacccctatttgtttatttttctaaatacattcaaatatgtatccgctcatgagacaataaccctgataaatgcttcaataatattgaaaaaggaagagtatgagtattcaacatttccgtgtcgcccttattcccttttttgcggcattttgccttcctgtttttgctcacccagaaacgctggtgaaagtaaaagatgctgaagatcagttgggtgcacgagtgggttacatcgaactggatctcaacagcggtaagatccttgagagttttcgccccgaagaacgttttccaatgatgagcacttttaaagttctgctatgtggcgcggtattatcccgtattgacgccgggcaagagcaactcggtcgccgcatacactattctcagaatgacttggttgagtactcaccagtcacagaaaagcatcttacggatggcatgacagtaagagaattatgcagtgctgccataaccatgagtgataacactgcggccaacttacttctgacaacgatcggaggaccgaaggagctaaccgcttttttgcacaacatgggggatcatgtaactcgccttgatcgttgggaaccggagctgaatgaagccataccaaacgacgagcgtgacaccacgatgcctgtagcaatggcaacaacgttgcgcaaactattaactggcgaactacttactctagcttcccggcaacaattaatagactggatggaggcggataaagttgcaggaccacttctgcgctcggcccttccggctggctggtttattgctgataaatctggagccggtgagcgtgggtctcgcggtatcattgcagcactggggccagatggtaagccctcccgtatcgtagttatctacacgacggggagtcaggcaactatggatgaacgaaatagacagatcgctgagataggtgcctcactgattaagcattggtaactgtcagaccaagtttactcatatatactttagattgatttaaaacttcatttttaatttaaaaggatctaggtgaagatcctttttgataatctcatgaccaaaatcccttaacgtgagttttcgttccactgagcgtcagaccccgtagaaaagatcaaaggatcttcttgagatcctttttttctgcgcgtaatctgctgcttgcaaacaaaaaaaccaccgctaccagcggtggtttgtttgccggatcaagagctaccaactctttttccgaaggtaactggcttcagcagagcgcagataccaaatactgttcttctagtgtagccgtagttaggccaccacttcaagaactctgtagcaccgcctacatacctcgctctgctaatcctgttaccagtggctgctgccagtggcgataagtcgtgtcttaccgggttggactcaagacgatagttaccggataaggcgcagcggtcgggctgaacggggggttcgtgcacacagcccagcttggagcgaacgacctacaccgaactgagatacctacagcgtgagctatgagaaagcgccacgcttcccgaagggagaaaggcggacaggtatccggtaagcggcagggtcggaacaggagagcgcacgagggagcttccagggggaaacgcctggtatctttatagtcctgtcgggtttcgccacctctgacttgagcgtcgatttttgtgatgctcgtcaggggggcggagcctatggaaaaacgccagcaacgcggcctttttacggttcctggccttttgctggccttttgctcacatgttctttcctgcgttatcccctgattctgtggataaccgtattaccgcctttgagtgagctgataccgctcgccgcagccgaacgaccgagcgcagcgagtcagtgagcgaggaagcggaagagcgcccaatacgcaaaccgcctctccccgcgcgttggccgattcattaatgcagctggcacgacaggtttcccgactggaaagcgggcagtgagcgcaacgcaattaatgtgagttagctcactcattaggcaccccaggctttacactttatgcttccggctcgtatgttgtgtggaattgtgagcggataacaatttcacacaggaaacagctatgaccatgattacgccaagctctagctagaggtcgacggtatacagacatgataagatacattgatgagtttggacaaaccacaactagaatgcagtgaaaaaaatgctttatttgtgaaatttgtgatgctattgctttatttgtaaccattataagctgcaataaacaagttggggtgggcgaagaactccagcatgagatccccgcgctggaggatcatccagccggcgtcccggaaaacgattccgaagcccaacctttcatagaaggcggcggtggaatcgaaatctcgtagtacgtgctattcctttgccctcggacgagtgctggggcgtcggtttccactatcggcgagtacttctacacagccatcggtccagacggccgcgcttctgcgggcgatttgtgtacgcccgacagtcccggctccggatcggacgattgcgtcgcatcgaccctgcgcccaagctgcatcatcgaaattgccgtcaaccaagctctgatagagttggtcaagaccaatgcggagcatatacgcccggagccgcggcgatcctgcaagctccggatgcctccgctcgaagtagcgcgtctgctgctccatacaagccaaccacggcctccagaagaagatgttggcgacctcgtattgggaatccccgaacatcgcctcgctccagtcaatgaccgctgttatgcggccattgtccgtcaggacattgttggagccgaaatccgcgtgcacgaggtgccggacttcggggcagtcctcggcccaaagcatcagctcatcgagagcctgcgcgacggacgcactgacggtgtcgtccatcacagtttgccagtgatacacatggggatcagcaatcgcgcatatgaaatcacgccatgtagtgtattgaccgattccttgcggtccgaatgggccgaacccgctcgtctggctaagatcggccgcagcgatcgcatccatggcctccgcgaccggctgcagaacagcgggcagttcggtttcaggcaggtcttgcaacgtgacaccctgtgcacggcgggagatgcaataggtcaggctctcgctgaattccccaatgtcaagcacttccggaatcgggagcgcggccgatgcaaagtgccgataaacataacgatctttgtagaaaccatcggcgcagctatttacccgcaggacatatccacgccctcctacatcgaagctgaaagcacgagattcttcgccctccgagagctgcatcaggtcggagacgctgtcgaacttttcgatcagaaacttctcgacagacgtcgcggtgagttcaggctttttggccaaggaagttcctatactttctagagaataggaacttcggaataggaacttctaggtacgtgaaccatcaccctaatcaagttttttggggtcgaggtgccgtaaagcactaaatcggaaccctaaagggagcccccgatttagagcttgacggggaaagccggcgaacgtggcgagaaaggaagggaagaaagcgaaaggagcgggcgctagggcgctggcaagtgtagcggtcacgctgcgcgtaaccaccacacccgccgcgcttaatgcgccgctacagggcgcgtggggataccccctagagccccagctggttctttccgcctcagaagccatagagcccaccgcatccccagcatgcgaacgaccgagcgcagcgagtcagtgagcgaggaagctcggggcagtgaaaaaaatgctttatttgtgaaatttgtgatgctattgctttatttgtaaccattataagctgcaataaacaagttaacaacaacaattgcattcattttatgtttcaggttcagggggaggtgtgggaggttttttaaagcaagtaaaacctctacaaatgtggtatggctgattatgatcctctggagatatcgtcgacaagcttatcgatgcggccgcgctagcttagcttgccgggggacagggacagggacttctgagtgtagtgattgtgcagggcctcgtgcatcacggagcaggagaacacgttgccctgctgccaacgggacttgtccacggtcagcttgctgtacaggaagaaggaaccgtcggagtccagcacgggaggggtggtcttgtagttgttctcgggctggccgttgctctcccattccacggcgatgtcggaggggtagaagcctttcaccaggcaggtgagggagacctggttcttggtcatctcctcgcggctgggaggcagagtgtacacctggggctcacgaggttggcccttagccttggagatggtcttctcgatgggagcgggcagggccttgttggacactttgcacttgtactccttgccgttcagccagtcctggtgcagcacggtgagcacggacacgacgcggtaggtgctgttgtactgctcctcacggggcttggtcttagcgttgtgcacctcgacgccgtccacgtaccagttgaacttcacctcggggtcctcgtgggacacatccaccacgacgcaagtcacctcgggagtgcgggagatcatcagggtgtccttgggcttgggagggaacagaaacacggaggggccaccgagcagttcaggagcagggcaaggggggcaagtgtgggtcttgtcgcaggacttgggctcgaccttcttgtccaccttggtgttggagggcttgtggttcacgttgcagatgtaggtctgggtgcccagggaggatgagggcacagtcacgacggaggacagggagtacaggccggaggactgcaggacagcagggaaggtgtgcacgccggaggtcagagcaccggagttccaagacacggtcacgggctcggggaagtagtccttgaccaggcaacccagagcagcggttccaccggaggtggacttggaggatggagccagagggaacacggaggggcccttggtggaagcagaggacacggtgaccagggtgccctggccccagtagtccatagcgtagaaaccgtcgccaccccaacgggagcagtagtacacagcggtgtcctcagcacgcagggagttcatctgcaggtaagcggtgttcttggaggtgtcagcggagatggtgaaacggcccttcacggagtcagcgtaacgggtgtaaccgttggtggggtagatacgggccacccattccaatcccttgccgggagcctggcggacccagtggatgtaggtgtccttgatgttgaaaccggaagcagcgcaggacagacgcagggaaccaccaggctgaaccaggccaccaccggactcgaccagctgcacttcggaataagccgagctaaagagaaaaagaagggaaataaaggttacccacttcatggtggcggatccctagcggatctgacggttcactaaaccagctctgcttatatagacctcccaccgtacacgcctaccgcccatttgcgtcaatggggcggagttgttacgacattttggaaagtcccgttgattttggtgccaaaacaaactcccattgacgtcaatggggtggagacttggaaatccccgtgagtcaaaccgctatccacgcccattgatgtactgccaaaaccgcatcaccatggtaatagcgatgactaatacgtagatgtactgccaagtaggaaagtcccataaggtcatgtactgggcataatgccaggcgggccatttaccgtcattgacgtcaatagggggcgtacttggcatatgatacacttgatgtactgccaagtgggcagtttaccgtaaatactccacccattgacgtcaatggaaagtccctattggcgttactatgggaacatacgtcattattgacgtcaatgggcgggggtcgttgggcggtcagccaggcgggccatttaccgtaagttatgtaacgcggaactccatatatgggctatgaactaatgaccccgtaattgattactattaataactactcgagtatgtcgaggtggcgtgtacggtgggaggcctatataagcagagctcgtttagtgaaccgtcagatcgcctggagaattcgccaccatgaagtgggtaacctttatttcccttctttttctctttagctcggcttattccgacatccagatgacccagtccccctcctccctgtccgcttccgtgggagatcgtgtgaccatcacttgccgtgcttcccaggacgtgaacaccgctgtggcttggtaccagcagaagcccggcaaggctcccaagctgctgatctactccgctagcttcctgtactccggtgtcccctcccgtttctccggttcccgttccggtactgacttcaccctgaccatctccagcctgcagcccgaggacttcgctacctactactgccagcagcactacaccaccccccccaccttcggccagggtactaaggtcgagatcaagcgtaccgtggctgctccctccgtgttcatcttcccaccctccgacgagcagctgaagtccggcactgcttccgtcgtgtgcctgctgaacaacttctacccccgcgaggctaaggtgcagtggaaggtggacaacgctctgcagtccggcaactcccaagagtccgtgaccgagcaggactccaaggactctacctactctctgtcctctaccctgaccctgtccaaggctgactacgagaagcacaaggtgtacgcttgcgaagtgacccaccagggcctgtcctccccagtgaccaagtccttcaaccgtggcgagtgctaaactagtggcgcgccgatcataatcagccataccacatttgtagaggttttacttgctttaaaaaacctcccacacctccccctgaacctgaaacataaaatgaatgcaattgttgttgttaacttgtttattgcagcttataatggttacaaataaagcaatagcatcacaaatttcacaaataaagcatttttttcactgccgacgtcaggtggcacttttcggacgcgtatatctggcccgtacatcgcgaagcagcgcaaaacgcctaaccctaagcagattcttcatgcaattgtcggtcaagccttgccttgttgtagcttaaattttgctcgcgcactactcagcgacctccaacacacaagcagggagcagatactggcttaactatgcggcatcagagcagattgtactgagagtgcaccataggggatcgggagatctcccgatccgtc

SEQ ID NO: 50 - protein, 902 aa, synthetic construct
  REGION 1..902: note = NLS-T7 Polymerase
  REGION 3..20: note = MISC_FEATURE - NLS
MGRLESTPPKKKRKVEDSASNTINIAKNDFSDIELAAIPFNTLADHYGERLAREQLALEHESYEMGEARFRKMFERQLKAGEVADNAAAKPLITTLLPKMIARINDWFEEVKAKRGKRPTAFQFLQEIKPEAVAYITIKTTLACLTSADNTTVQAVASAIGRAIEDEARFGRIRDLEAKHFKKNVEEQLNKRVGHVYKKAFMQVVEADMLSKGLLGGEAWSSWHKEDSIHVGVRCIEMLIESTGMVSLHRQNAGVVGQDSETIELAPEYAEAIATRAGALAGISPMFQPCVVPPKPWTGITGGGYWANGRRPLALVRTHSKKALMRYEDVYMPEVYKAINIAQNTAWKINKKVLAVANVITKWKHCPVEDIPAIEREELPMKPEDIDMNPEALTAWKRAAAAVYRKDKARKSRRISLEFMLEQANKFANHKAIWFPYNMDWRGRVYAVSMFNPQGNDMTKGLLTLAKGKPIGKEGYYWLKIHGANCAGVDKVPFPERIKFIEENHENIMACAKSPLENTWWAEQDSPFCFLAFCFEYAGVQHHGLSYNCSLPLAFDGSCSGIQHFSAMLRDEVGGRAVNLLPSETVQDIYGIVAKKVNEILQADAINGTDNEVVTVTDENTGEISEKVKLGTKALAGQWLAYGVTRSVTKRSVMTLAYGSKEFGFRQQVLEDTIQPAIDSGKGLMFTQPNQAAGYMAKLIWESVSVTVVAAVEAMNWLKSAAKLLAAEVKDKKTGEILRKRCAVHWVTPDGFPVWQEYKKPIQTRLNLMFLGQFRLQPTINTNKDSEIDAHKQESGIAPNFVHSQDGSHLRKTVVWAHEKYGIESFALIHDSFGTIPADAANLFKAVRETMVDTYESCDVLADFYDQFADQLHESQLDKMPALPAKGNLNLRDILESDFAFA

SEQ ID NO: 51 - protein, 218 aa, synthetic construct
  REGION 1..218: note = TetRepressor
MSRLDKSKVINSALELLNEVGIEGLTTRKLAQKLGVEQPTLYWHVKNKRALLDALAIEMLDRHHTHFCPLEGESWQDFLRNNAKSFRCALLSHRDGAKVHLGTRPTEKQYETLENQLAFLCQQGFSLENALYALSAVGHFTLGCVLEDQEHQVAKEERETPTTDSMPPLLRQAIELFDHQGAEPAFLFGLELIICGLEKQLKCESGSAYSGSREFRSY

SEQ ID NO: 52 - protein, 471 aa, synthetic construct
  REGION 1..471: note = NES-PylRS A1 mutant
  REGION 2..18: note = MISC_FEATURE - NES
MACPVPLQLPPLERLTLDDKKPLNTLISATGLWMSRTGTIHKIKHHEVSRSKIYIEMACGDHLVVNNSRSSRTARALRHHKYRKTCKRCRVSDEDLNKFLTKANEDQTSVKVKVVSAPTRTKKAMPKSVARAPKPLENTEAAQAQPSGSKFSPAIPVSTQESVSVPASVSTSISSISTGATASALVKGNTNPITSMSAPVQASAPALTKSQTDRLEVLLNPKDEISLNSGKPFRELESELLSRRKKDLQQIYAEERENYLGKLEREITRFFVDRGFLEIKSPILIPLEYIERMGIDNDTELSKQIFRVDKNFCLRPMLAPNLYNYMRKLDRALPDPIKIFEIGPCYRKESDGKEHLEEFTMLNFGQMGSGCTRENLESIITDFLNHLGIDFKIVGDSCMVYGDTLDVMHGDLELSSAVVGPRPLDREWGIDKPWIGAGFGLERLLKVKHDFKNIKRAARSESYYNGISTNL

SEQ ID NO: 53 - protein, 183 aa, synthetic construct
  REGION 1..183: note = Protein KinaseR deletion mutant
  REGION 2..10: note = MISC_FEATURE - HA signal
MYPYDVPDYAAGDLSAGFFMEELNTYRQKQGVVLKYQELPNSGPPHDRRFTFQVIIDGREFPEGEGRSKKEAKNAAAKLAVEILNKEKKAVSPLLLTTTNSSEGLSMGNYIGLINRIAQKKRLTVNYEQCASGVHGPEGFHYKCKMGQKEYSIGTGSTKQEAKQLAAKLAYLQILSEETSVKS

SEQ ID NO: 54 - DNA, 295 bp, synthetic construct
  misc_feature 1..295: note = Expression construct
  source 1..295: mol_type = other DNA
taatacgactcactataggaaacctgatcatgtagatcgaatggactctaaatccgttcagccgggttagattcccggggtttccggctagccatggtcccagcctcctcgctggcggctagtgggcaacatgcttcggcatggcgaatgggactttaaactcgagctgctaacaaagcccgaaaggaagctgagttggctgctgccaccgctgagcaataactagcataaccccttggggcctctaaacgggtcttgaggggttttttgctgaaaggaggaactatatccggat

SEQ ID NO: 55 - DNA, 26 bp, synthetic construct
  misc_feature 1..26: note = PCR primer
  source 1..26: mol_type = other DNA
tcctcttagtccaccaagggcccctc

SEQ ID NO: 56 - DNA, 29 bp, synthetic construct
  misc_feature 1..29: note = PCR primer
  source 1..29: mol_type = other DNA
ggtggactaagaggacacggtgaccaggg

SEQ ID NO: 57 - DNA, 41 bp, synthetic construct
  misc_feature 1..41: note = PCR primer
  source 1..41: mol_type = other DNA
ctgcgctgcatagggcttcaacatcaaggacacctacatcc

SEQ ID NO: 58 - DNA, 34 bp, synthetic construct
  misc_feature 1..34: note = PCR primer
  source 1..34: mol_type = other DNA
gaagccctatgcagcgcagctcagtctcagactc

SEQ ID NO: 59 - DNA, 41 bp, synthetic construct
  misc_feature 1..41: note = PCR primer
  source 1..41: mol_type = other DNA
agcccctggatagggcttggagtgggtggctagaatctacc

SEQ ID NO: 60 - DNA, 37 bp, synthetic construct
  misc_feature 1..37: note = PCR primer
  source 1..37: mol_type = other DNA
actccaagccctatccaggggcttgtctcacccagtg

SEQ ID NO: 61 - DNA, 36 bp, synthetic construct
  misc_feature 1..36: note = PCR primer
  source 1..36: mol_type = other DNA
gtgggttgcatagatctaccccaccaacggctacac

SEQ ID NO: 62 - DNA, 31 bp, synthetic construct
  misc_feature 1..31: note = PCR primer
  source 1..31: mol_type = other DNA
gtagatctatgcaacccactccaggcccttg

SEQ ID NO: 63 - DNA, 44 bp, synthetic construct
  misc_feature 1..44: note = PCR primer
  source 1..44: mol_type = other DNA
agcctgcgtgcataggacacggccgtgtactactgcagcagatg

SEQ ID NO: 64 - DNA, 44 bp, synthetic construct
  misc_feature 1..44: note = PCR primer
  source 1..44: mol_type = other DNA
cacggccgtgtcctatgcacgcaggctgttcatctgcaggtagg

SEQ ID NO: 65 - DNA, 41 bp, synthetic construct
  misc_feature 1..41: note = PCR primer
  source 1..41: mol_type = other DNA
gccgactctgtatagggcaggttcaccatcagcgccgacac

SEQ ID NO: 66 - DNA, 43 bp, synthetic construct
  misc_feature 1..43: note = PCR primer
  source 1..43: mol_type = other DNA
ggtgaacctgccctatacagagtcggcgtatcttgtgtagccg

SEQ ID NO: 67 - DNA, 39 bp, synthetic construct
  misc_feature 1..39: note = PCR primer
  source 1..39: mol_type = other DNA
aagatatgcatagtccgtgaagggcagattcaccatcag

SEQ ID NO: 68 - DNA, 39 bp, synthetic construct
  misc_feature 1..39: note = PCR Sequence
  source 1..39: mol_type = other DNA
ttcacggactatgcatatcttgtgtagccgttggtgggg

SEQ ID NO: 69 - DNA, 37 bp, synthetic construct
  misc_feature 1..37: note = PCR primer
  source 1..37: mol_type = other DNA
atggggtggatagggcttctacgccatggactactgg

SEQ ID NO: 70 - DNA, 37 bp, synthetic construct
  misc_feature 1..37: note = PCR primer
  source 1..37: mol_type = other DNA
gaagccctatccaccccatctgctgcagtagtacacg

SEQ ID NO: 71 - DNA, 33 bp, synthetic construct
  misc_feature 1..33: note = PCR primer
  source 1..33: mol_type = other DNA
ttttccatagcccgtgaccgtcagttggaattc

SEQ ID NO: 72 - DNA, 37 bp, synthetic construct
  misc_feature 1..37: note = PCR primer
  source 1..37: mol_type = other DNA
cacgggctatggaaaataatccttcactaggcagccc

SEQ ID NO: 73 - DNA, 39 bp, synthetic construct
  misc_feature 1..39: note = PCR primer
  source 1..39: mol_type = other DNA
ttttcctgaataggtcacggtcagttggaattccggcgc

SEQ ID NO: 74 - DNA, 48 bp, synthetic construct
  misc_feature 1..48: note = PCR primer
  source 1..48: mol_type = other DNA
actgaccgtgacctattcaggaaaataatccttcactaggcagcccag

SEQ ID NO: 75 - DNA, 39 bp, synthetic construct
  misc_feature 1..39: note = PCR primer
  source 1..39: mol_type = other DNA
gtgccttcatagtccttgggcacacagacctacatctgc

SEQ ID NO: 76 - DNA, 33 bp, synthetic construct
  misc_feature 1..33: note = PCR primer
  source 1..33: mol_type = other DNA
tgcccaaggactatgaaggcacggtcaccacgc

SEQ ID NO: 77 - DNA, 40 bp, synthetic construct
  misc_feature 1..40: note = PCR primer
  source 1..40: mol_type = other DNA
caagaaagtatagcccaagagctgtgacaagacccacacc

SEQ ID NO: 78 - DNA, 42 bp, synthetic construct
  misc_feature 1..42: note = PCR primer
  source 1..42: mol_type = other DNA
gctcttgggctatactttcttgtccaccttggtgttgctagg

SEQ ID NO: 79 - DNA, 40 bp, synthetic construct
  misc_feature 1..40: note = PCR primer
  source 1..40: mol_type = other DNA
caagcctaaatagaccttgatgatcagcagaacccccgag

SEQ ID NO: 80 - DNA, 40 bp, synthetic construct
  misc_feature 1..40: note = PCR primer
  source 1..40: mol_type = other DNA
tcatcaaggtctatttaggcttggggggaaaaaggaacac

SEQ ID NO: 81 - DNA, 40 bp, synthetic construct
  misc_feature 1..40: note = PCR primer
  source 1..40: mol_type = other DNA
cgaggatccataggtcaagttcaactggtacgtggacggc

SEQ ID NO: 82 - DNA, 36 bp, synthetic construct
  misc_feature 1..36: note = PCR primer
  source 1..36: mol_type = other DNA
gaacttgacctatggatcctcgtggctcacgtccac

SEQ ID NO: 83 - DNA, 34 bp, synthetic construct
  misc_feature 1..34: note = PCR primer
  source 1..34: mol_type = other DNA
ccccgaagtatagttcaactggtacgtggacggc

SEQ ID NO: 84 - DNA, 27 bp, synthetic construct
  misc_feature 1..27: note = PCR primer
  source 1..27: mol_type = other DNA
tgaactatacttcggggtcctcgtggc

SEQ ID NO: 85 - DNA, 31 bp, synthetic construct
  misc_feature 1..31: note = PCR primer
  source 1..31: mol_type = other DNA
ctggtatgtatagggcgtggaggtgcacaac

SEQ ID NO: 86 - DNA, 37 bp, synthetic construct
  misc_feature 1..37: note = PCR primer
  source 1..37: mol_type = other DNA
cacgccctatacataccagttgaacttcacctcgggg

SEQ ID NO: 87 - DNA, 43 bp, synthetic construct
  misc_feature 1..43: note = PCR primer
  source 1..43: mol_type = other DNA
cgtggaagtatagaacgcgaagaccaagcctagagaggagcag

SEQ ID NO: 88 - DNA, 37 bp, synthetic construct
  misc_feature 1..37: note = PCR primer
  source 1..37: mol_type = other DNA
ggtcttcgcgttctatacttccacgccgtccacgtac

SEQ ID NO: 89 - DNA, 45 bp, synthetic construct
  misc_feature 1..45: note = PCR primer
  source 1..45: mol_type = other DNA
cgccaaaacatagcccagggaggagcagtacaacagcacctacag

SEQ ID NO: 90 - DNA, 39 bp, synthetic construct
  misc_feature 1..39: note = PCR primer
  source 1..39: mol_type = other DNA
ctcctccctgggctatgttttggcgttgtgcacctccac

SEQ ID NO: 91 - DNA, 39 bp, synthetic construct
  misc_feature 1..39: note = PCR primer
  source 1..39: mol_type = other DNA
aagcctcgataggagcagtacaacagcacctacagagtg

SEQ ID NO: 92 - DNA, 33 bp, synthetic construct
  misc_feature 1..33: note = PCR primer
  source 1..33: mol_type = other DNA
ctgctcctatcgaggcttggtcttggcgttgtg

SEQ ID NO: 93 - DNA, 35 bp, synthetic construct
  misc_feature 1..35: note = PCR primer
  source 1..35: mol_type = other DNA
cagcacttactaggtcgtgagcgtgctgaccgtgc

SEQ ID NO: 94 - DNA, 42 bp, synthetic construct
  misc_feature 1..42: note = PCR primer
  source 1..42: mol_type = other DNA
gctcacgacctagtaagtgctgttgtactgctcctctctagg

SEQ ID NO: 95 - DNA, 33 bp, synthetic construct
  misc_feature 1..33: note = PCR primer
  source 1..33: mol_type = other DNA
caaggaatactagtgcaaggtgagcaacaaggc

SEQ ID NO: 96 - DNA, 31 bp, synthetic construct
  misc_feature 1..31: note = PCR primer
  source 1..31: mol_type = other DNA
tgcactagtattccttgccgttcagccagtc

SEQ ID NO: 97 - DNA, 43 bp, synthetic construct
  misc_feature 1..43: note = PCR primer
  source 1..43: mol_type = other DNA
gaagcctggataggccccgaagctgctgatctacagcgcaagc

SEQ ID NO: 98 - DNA, 40 bp, synthetic construct
  misc_feature 1..40: note = PCR primer
  source 1..40: mol_type = other DNA
cagcttcggggcctatccaggcttctgctgataccaggcc

SEQ ID NO: 99 - DNA, 43 bp, synthetic construct
  misc_feature 1..43: note = PCR primer
  source 1..43: mol_type = other DNA
caaggctccatagctcttgatctacagcgcaagcttcctgtac

SEQ ID NO: 100 - DNA, 34 bp, synthetic construct
  misc_feature 1..34: note = PCR primer
  source 1..34: mol_type = other DNA
agatcaagagctatggagccttgccgggcttctg

SEQ ID NO: 101 - DNA, 35 bp, synthetic construct
  misc_feature 1..35: note = PCR primer
  source 1..35: mol_type = other DNA
gtgccttcatagttctcgggcagcagaagcggcac

SEQ ID NO: 102 - DNA, 36 bp, synthetic construct
  misc_feature 1..36: note = PCR primer
  source 1..36: mol_type = other DNA
gctgcccgagaactatgaaggcacgccgctgtacag

SEQ ID NO: 103 - DNA, 40 bp, synthetic construct
  misc_feature 1..40: note = PCR primer
  source 1..40: mol_type = other DNA
aagcggtacatagttcacgctgaccatcagcagcctgcag

SEQ ID NO: 104 - DNA, 35 bp, synthetic construct
  misc_feature 1..35: note = PCR primer
  source 1..35: mol_type = other DNA
ggtcagcgtgaactatgtaccgcttctgctgccgc

SEQ ID NO: 105 - DNA, 37 bp, synthetic construct
  misc_feature 1..37: note = PCR primer
  source 1..37: mol_type = other DNA
cctgcaaccataggacttcgccacctactactgtcag

SEQ ID NO: 106 - DNA, 31 bp, synthetic construct
  misc_feature 1..31: note = PCR primer
  source 1..31: mol_type = other DNA
agtcctatggttgcaggctgctgatggtcag

SEQ ID NO: 107 - DNA, 30 bp, synthetic construct
  misc_feature 1..30: note = PCR primer
  source 1..30: mol_type = other DNA
taccctcgataggccaaggtgcagtggaag

SEQ ID NO: 108 - DNA, 35 bp, synthetic construct
  misc_feature 1..35: note = PCR primer
  source 1..35: mol_type = other DNA
tggcctatcgagggtagaagttgttcagcaggcac

SEQ ID NO: 109 - DNA, 37 bp, synthetic construct
  misc_feature 1..37: note = PCR primer
  source 1..37: mol_type = other DNA
gtggaaagtatagaacgcgctgcagagcggcaacagc

SEQ ID NO: 110 - DNA, 39 bp, synthetic construct
  misc_feature 1..39: note = PCR primer
  source 1..39: mol_type = other DNA
ctgcagcgcgttctatactttccactgcaccttggcctc

SEQ ID NO: 111 - DNA, 41 bp, synthetic construct
  misc_feature 1..41: note = PCR primer
  source 1..41: mol_type = other DNA
cctgcaatcatagaactcgcaagagagcgtgaccgagcaag

SEQ ID NO: 112 - DNA, 37 bp, synthetic construct
  misc_feature 1..37: note = PCR primer
  source 1..37: mol_type = other DNA
ctcttgcgagttctatgattgcagggcgttgtccacc

SEQ ID NO: 113 - DNA, 37 bp, synthetic construct
  misc_feature 1..37: note = PCR primer
  source 1..37: mol_type = other DNA
gacccatcaatagctctcgagccccgtgaccaagagc

SEQ ID NO: 114 - DNA, 36 bp, synthetic construct
  misc_feature 1..36: note = PCR primer
  source 1..36: mol_type = other DNA
ggggctcgagagctattgatgggtcacctcgcaggc

SEQ ID NO: 115 - DNA, 25 bp, synthetic construct
  source 1..25: mol_type = other DNA
  misc_feature 1..25: note = PCR primer
aacgcttagaccaagccccgtgagg

SEQ ID NO: 116 - DNA, 26 bp, synthetic construct
  source 1..26: mol_type = other DNA
  misc_feature 1..26: note = PCR primer
tggtctaagcgttgtgcacctcgacg